European Patent Application EP 4 653 016 A1, published November 26, 2025. Title: CONJUGATE OF ERIBULIN DRUG. Applicant: SYSTIMMUNE, INC. Application EP 24744298.1, filed January 17, 2024. The sequence listing filed with the application follows.

SEQUENCE LISTING (30 sequences)

SEQ ID NO: 1 - protein, 11 aa, synthetic construct
RASQDINKYLA

SEQ ID NO: 2 - protein, 7 aa, synthetic construct
STSTLQS

SEQ ID NO: 3 - protein, 8 aa, synthetic construct
LQYDDLFT

SEQ ID NO: 4 - protein, 5 aa, synthetic construct
SFDIN

SEQ ID NO: 5 - protein, 17 aa, synthetic construct
WIFPGDGNTKYSQKFQG

SEQ ID NO: 6 - protein, 9 aa, synthetic construct
GEALYYFDY

SEQ ID NO: 7 - protein, 106 aa, synthetic construct
DIQMTQSPSSLSASVGDRVTITCRASQDINKYLAWYQQKPGKVPKLLIYSTSTLQSGVPSRFSGSGSGTDFTLTISSLQPEDVATYYCLQYDDLFTFGQGTKLEIK

SEQ ID NO: 8 - protein, 107 aa, synthetic construct [sequence omitted]

SEQ ID NO: 9 - protein, 213 aa, synthetic construct
DIQMTQSPSSLSASVGDRVTITCRASQDINKYLAWYQQKPGKVPKLLIYSTSTLQSGVPSRFSGSGSGTDFTLTISSLQPEDVATYYCLQYDDLFTFGQGTKLEIKRTVAAPSVFIFPPSDEQLKSGTASVVCLLNNFYPREAKVQWKVDNALQSGNSQESVTEQDSKDSTYSLSSTLTLSKADYEKHKVYACEVTHQGLSSPVTKSFNRGEC

SEQ ID NO: 10 - protein, 106 aa, synthetic construct; identical to SEQ ID NO: 7

SEQ ID NO: 11 - protein, 108 aa, synthetic construct
RTVAAPSVFIFPPSDEQLKSGTASVVCLLNNFYPREAKVQWKVDNALQSGNSQESVTEQDSKDSTYSLSSTLTLSKADYEKHKVYACEVTHQGLSSPVCTKSFNRGEC

SEQ ID NO: 12 - protein, 214 aa, synthetic construct
DIQMTQSPSSLSASVGDRVTITCRASQDINKYLAWYQQKPGKVPKLLIYSTSTLQSGVPSRFSGSGSGTDFTLTISSLQPEDVATYYCLQYDDLFTFGQGTKLEIKRTVAAPSVFIFPPSDEQLKSGTASVVCLLNNFYPREAKVQWKVDNALQSGNSQESVTEQDSKDSTYSLSSTLTLSKADYEKHKVYACEVTHQGLSSPVCTKSFNRGEC

SEQ ID NO: 13 - protein, 118 aa, synthetic construct
QVQLVQSGAEVKKPGASVKLSCKASGYTFTSFDINWVRQAPEQRLEWMGWIFPGDGNTKYSQKFQGRATITRDTSASTAYMELSSLRSEDTAVYYCVRGEALYYFDYWGQGTLVTVSS

SEQ ID NO: 14 - protein, 329 aa, synthetic construct
ASTKGPSVFPLAPSSKSTSGGTAALGCLVKDYFPEPVTVSWNSGALTSGVHTFPAVLQSSGLYSLSSVVTVPSSSLGTQTYICNVNHKPSNTKVDKRVEPKSCDKTHTCPPCPAPELLGGPSVFLFPPKPKDTLMISRTPEVTCVVVDVSHEDPEVKFNWYVDGVEVHNAKTKPREEQYNSTYRVVSVLTVLHQDWLNGKEYKCKVSNKALPAPIEKTISKAKGQPREPQVYTLPPSRDELTKNQVSLTCLVKGFYPSDIAVEWESNGQPENNYKTTPPVLDSDGSFFLYSKLTVDKSRWQQGNVFSCSVMHEALHNHYTQKSLSLSPG

SEQ ID NO: 15 - protein, 447 aa, synthetic construct
QVQLVQSGAEVKKPGASVKLSCKASGYTFTSFDINWVRQAPEQRLEWMGWIFPGDGNTKYSQKFQGRATITRDTSASTAYMELSSLRSEDTAVYYCVRGEALYYFDYWGQGTLVTVSSASTKGPSVFPLAPSSKSTSGGTAALGCLVKDYFPEPVTVSWNSGALTSGVHTFPAVLQSSGLYSLSSVVTVPSSSLGTQTYICNVNHKPSNTKVDKRVEPKSCDKTHTCPPCPAPELLGGPSVFLFPPKPKDTLMISRTPEVTCVVVDVSHEDPEVKFNWYVDGVEVHNAKTKPREEQYNSTYRVVSVLTVLHQDWLNGKEYKCKVSNKALPAPIEKTISKAKGQPREPQVYTLPPSRDELTKNQVSLTCLVKGFYPSDIAVEWESNGQPENNYKTTPPVLDSDGSFFLYSKLTVDKSRWQQGNVFSCSVMHEALHNHYTQKSLSLSPG

SEQ ID NO: 16 - DNA, 33 bp, synthetic construct
  source 1..33: mol_type = other DNA
agagcttctcaggatatcaataagtatctggct

SEQ ID NO: 17 - DNA, 21 bp, synthetic construct
  source 1..21: mol_type = other DNA
tctacatctaccctgcagtct

SEQ ID NO: 18 - DNA, 24 bp, synthetic construct
  source 1..24: mol_type = other DNA
ctgcagtatgatgatctgttcacc

SEQ ID NO: 19 - DNA, 15 bp, synthetic construct
  source 1..15: mol_type = other DNA
tccttcgacattaac

SEQ ID NO: 20 - DNA, 51 bp, synthetic construct
  source 1..51: mol_type = other DNA
tggatcttccccggcgacggcaacaccaagtactcccagaagttccaggga

SEQ ID NO: 21 - DNA, 27 bp, synthetic construct
  source 1..27: mol_type = other DNA
ggagaggctctgtactattttgattat

SEQ ID NO: 22 - DNA, 318 bp, synthetic construct
  source 1..318: mol_type = other DNA
gatatccagatgacccagtctccatctagcctgtccgcttctgtgggcgatagagtgaccatcacatgcagagcttctcaggatatcaataagtatctggcttggtatcagcagaagcctggaaaggtgcctaagctgctgatctactctacatctaccctgcagtctggagtgccttctagattttctggatctggctctggcaccgattttacactgacaatctcttctctgcagcctgaggatgtggctacatattattgtctgcagtatgatgatctgttcacctttggccagggcaccaagctggagatcaag

SEQ ID NO: 23 - DNA, 324 bp, synthetic construct
  source 1..324: mol_type = other DNA
cgtacggtggctgcaccatctgtcttcatcttcccgccatctgatgagcagttgaaatctggaactgcctctgttgtgtgcctgctgaataacttctatcccagagaggccaaagtacagtggaaggtggataacgccctccaatcgggtaactcccaggagagtgtcacagagcaggacagcaaggacagcacctacagcctcagcagcaccctgacgctgagcaaagcagactacgagaaacacaaagtctacgcctgcgaagtcacccatcagggcctgagctcgcccgtcacaaagagcttcaacaggggagagtgttag

SEQ ID NO: 24 - DNA, 642 bp, synthetic construct
  source 1..642: mol_type = other DNA
gatatccagatgacccagtctccatctagcctgtccgcttctgtgggcgatagagtgaccatcacatgcagagcttctcaggatatcaataagtatctggcttggtatcagcagaagcctggaaaggtgcctaagctgctgatctactctacatctaccctgcagtctggagtgccttctagattttctggatctggctctggcaccgattttacactgacaatctcttctctgcagcctgaggatgtggctacatattattgtctgcagtatgatgatctgttcacctttggccagggcaccaagctggagatcaagcgtacggtggctgcaccatctgtcttcatcttcccgccatctgatgagcagttgaaatctggaactgcctctgttgtgtgcctgctgaataacttctatcccagagaggccaaagtacagtggaaggtggataacgccctccaatcgggtaactcccaggagagtgtcacagagcaggacagcaaggacagcacctacagcctcagcagcaccctgacgctgagcaaagcagactacgagaaacacaaagtctacgcctgcgaagtcacccatcagggcctgagctcgcccgtcacaaagagcttcaacaggggagagtgttag

SEQ ID NO: 25 - DNA, 318 bp, synthetic construct; identical to SEQ ID NO: 22
  source 1..318: mol_type = other DNA

SEQ ID NO: 26 - DNA, 327 bp, synthetic construct
  source 1..327: mol_type = other DNA
cgtacggtggctgcaccatctgtcttcatcttcccgccatctgatgagcagttgaaatctggaactgcctctgttgtgtgcctgctgaataacttctatcccagagaggccaaagtacagtggaaggtggataacgccctccaatcgggtaactcccaggagagtgtcacagagcaggacagcaaggacagcacctacagcctcagcagcaccctgacgctgagcaaagcagactacgagaaacacaaagtctacgcctgcgaagtcacccatcagggcctgagctcgcccgtctgtacaaagagcttcaacaggggagagtgttag

SEQ ID NO: 27 - DNA, 645 bp, synthetic construct
  source 1..645: mol_type = other DNA
gatatccagatgacccagtctccatctagcctgtccgcttctgtgggcgatagagtgaccatcacatgcagagcttctcaggatatcaataagtatctggcttggtatcagcagaagcctggaaaggtgcctaagctgctgatctactctacatctaccctgcagtctggagtgccttctagattttctggatctggctctggcaccgattttacactgacaatctcttctctgcagcctgaggatgtggctacatattattgtctgcagtatgatgatctgttcacctttggccagggcaccaagctggagatcaagcgtacggtggctgcaccatctgtcttcatcttcccgccatctgatgagcagttgaaatctggaactgcctctgttgtgtgcctgctgaataacttctatcccagagaggccaaagtacagtggaaggtggataacgccctccaatcgggtaactcccaggagagtgtcacagagcaggacagcaaggacagcacctacagcctcagcagcaccctgacgctgagcaaagcagactacgagaaacacaaagtctacgcctgcgaagtcacccatcagggcctgagctcgcccgtctgtacaaagagcttcaacaggggagagtgttag

SEQ ID NO: 28 - DNA, 354 bp, synthetic construct
  source 1..354: mol_type = other DNA
caggtgcagctggtgcagtccggcgccgaggtgaagaagcccggcgcctccgtgaagctgagctgtaaggcctccggctacaccttcacctccttcgacattaactgggtgcggcaggcccccgagcagcgcctggagtggatgggctggatcttccccggcgacggcaacaccaagtactcccagaagttccagggaagagctaccatcaccagagatacatccgcttctacagcttacatggagctgtctagcctgagatctgaggatacagctgtgtattactgtgtgagaggagaggctctgtactattttgattattggggccagggcaccctggtgacagtgtcttct

SEQ ID NO: 29 - DNA, 990 bp, synthetic construct
  source 1..990: mol_type = other DNA
gctagcaccaagggcccatcggtcttccccctggcaccctcctccaagagcacctctgggggcacagcggccctgggctgcctggtcaaggactacttccccgaaccggtgacggtgtcgtggaactcaggcgccctgaccagcggcgtgcacaccttcccggctgtcctacagtcctcaggactctactccctcagcagcgtggtgaccgtgccctccagcagcttgggcacccagacctacatctgcaacgtgaatcacaagcccagcaacaccaaggtggacaagagagttgagcccaaatcttgtgacaaaactcacacatgcccaccgtgcccagcacctgaactcctggggggaccgtcagtcttcctcttccccccaaaacccaaggacaccctcatgatctcccggacccctgaggtcacatgcgtggtggtggacgtgagccacgaagaccctgaggtcaagttcaactggtacgtggacggcgtggaggtgcataatgccaagacaaagccgcgggaggagcagtacaacagcacgtaccgtgtggtcagcgtcctcaccgtcctgcaccaggactggctgaatggcaaggagtacaagtgcaaggtctccaacaaagccctcccagcccccatcgagaaaaccatctccaaagccaaagggcagccccgagaaccacaggtgtacaccctgcccccatcccgggatgagctgaccaagaaccaggtcagcctgacctgcctggtcaaaggcttctatcccagcgacatcgccgtggagtgggagagcaatgggcagccggagaacaactacaagaccacgcctcccgtgctggactccgacggctccttcttcctctatagcaagctcaccgtggacaagagcaggtggcagcaggggaacgtcttctcatgctccgtgatgcatgaggctctgcacaaccactacacgcagaagagcctctccctgtctccgggttaa

SEQ ID NO: 30 - DNA, 1344 bp, synthetic construct
  source 1..1344: mol_type = other DNA
caggtgcagctggtgcagtccggcgccgaggtgaagaagcccggcgcctccgtgaagctgagctgtaaggcctccggctacaccttcacctccttcgacattaactgggtgcggcaggcccccgagcagcgcctggagtggatgggctggatcttccccggcgacggcaacaccaagtactcccagaagttccagggaagagctaccatcaccagagatacatccgcttctacagcttacatggagctgtctagcctgagatctgaggatacagctgtgtattactgtgtgagaggagaggctctgtactattttgattattggggccagggcaccctggtgacagtgtcttctgctagcaccaagggcccatcggtcttccccctggcaccctcctccaagagcacctctgggggcacagcggccctgggctgcctggtcaaggactacttccccgaaccggtgacggtgtcgtggaactcaggcgccctgaccagcggcgtgcacaccttcccggctgtcctacagtcctcaggactctactccctcagcagcgtggtgaccgtgccctccagcagcttgggcacccagacctacatctgcaacgtgaatcacaagcccagcaacaccaaggtggacaagagagttgagcccaaatcttgtgacaaaactcacacatgcccaccgtgcccagcacctgaactcctggggggaccgtcagtcttcctcttccccccaaaacccaaggacaccctcatgatctcccggacccctgaggtcacatgcgtggtggtggacgtgagccacgaagaccctgaggtcaagttcaactggtacgtggacggcgtggaggtgcataatgccaagacaaagccgcgggaggagcagtacaacagcacgtaccgtgtggtcagcgtcctcaccgtcctgcaccaggactggctgaatggcaaggagtacaagtgcaaggtctccaacaaagccctcccagcccccatcgagaaaaccatctccaaagccaaagggcagccccgagaaccacaggtgtacaccctgcccccatcccgggatgagctgaccaagaaccaggtcagcctgacctgcctggtcaaaggcttctatcccagcgacatcgccgtggagtgggagagcaatgggcagccggagaacaactacaagaccacgcctcccgtgctggactccgacggctccttcttcctctatagcaagctcaccgtggacaagagcaggtggcagcaggggaacgtcttctcatgctccgtgatgcatgaggctctgcacaaccactacacgcagaagagcctctccctgtctccgggttaa